European Patent Application EP 4 534 698 A1, published April 9, 2025. Title: Serum microRNA markers associated with liver cancer and a new method for diagnosing liver cancer. Applicant: Qingdao Ruiside Medical Laboratory Co., Ltd. Application EP. The sequence listing filed with the application follows.

SEQUENCE LISTING (31 sequences)

SEQ ID NO: 1 - RNA, 23 nt, synthetic construct
  source 1..23: mol_type = other RNA; note = hsa-miR-107
agcagcattgtacagggctatca

SEQ ID NO: 2 - RNA, 22 nt, synthetic construct
  source 1..22: mol_type = other RNA; note = hsa-miR-122
tggagtgtgacaatggtgtttg

SEQ ID NO: 3 - RNA, 19 nt, synthetic construct
  source 1..19: mol_type = other RNA; note = hsa-miR-1246
aatggatttttggagcagg

SEQ ID NO: 4 - RNA, 21 nt, synthetic construct
  source 1..21: mol_type = other RNA; note = hsa-miR-192
ctgacctatgaattgacagcc

SEQ ID NO: 5 - RNA, 22 nt, synthetic construct
  source 1..22: mol_type = other RNA; note = hsa-miR-199
acagtagtctgcacattggtta

SEQ ID NO: 6 - RNA, 22 nt, synthetic construct
  source 1..22: mol_type = other RNA; note = hsa-miR-21
tagcttatcagactgatgttga

SEQ ID NO: 7 - RNA, 22 nt, synthetic construct
  source 1..22: mol_type = other RNA; note = hsa-miR-2115
catcagaattcatggaggctag

SEQ ID NO: 8 - RNA, 23 nt, synthetic construct
  source 1..23: mol_type = other RNA; note = hsa-miR-221
agctacattgtctgctgggtttc

SEQ ID NO: 9 - RNA, 22 nt, synthetic construct
  source 1..22: mol_type = other RNA; note = hsa-miR-223
tgtcagtttgtcaaatacccca

SEQ ID NO: 10 - RNA, 22 nt, synthetic construct
  source 1..22: mol_type = other RNA; note = hsa-miR-26
ttcaagtaatccaggataggct

SEQ ID NO: 11 - RNA, 21 nt, synthetic construct
  source 1..21: mol_type = other RNA; note = hsa-miR-27
ttcacagtggctaagttccgc

SEQ ID NO: 12 - RNA, 24 nt, synthetic construct
  source 1..24: mol_type = other RNA; note = hsa-miR-4499
gattgctctgcgtgcggaatcgac

SEQ ID NO: 13 - RNA, 22 nt, synthetic construct
  source 1..22: mol_type = other RNA; note = hsa-miR-801
gattgctgcgtgcggaatcgac

SEQ ID NO: 14 - RNA, 106 nt, synthetic construct
  source 1..106: mol_type = other RNA; note = RNU6-1
gtgctcgcttcggcagcacatatactaaaattggaacgatacagagaagattagcatggcccctgcgcaaggatgacacgcaaattcgtgaagcgttccatatttt

SEQ ID NO: 15 - DNA, 23 bp, synthetic construct
  source 1..23: mol_type = other DNA; note = hsa-miR-107-F
aacaagagcagcattgtacaggg

SEQ ID NO: 16 - DNA, 21 bp, synthetic construct
  source 1..21: mol_type = other DNA; note = hsa-miR-122-F
gccgagtggagtgtgacaatg

SEQ ID NO: 17 - DNA, 23 bp, synthetic construct
  source 1..23: mol_type = other DNA; note = hsa-miR-1246-F
aacacgcaatggatttttggagc

SEQ ID NO: 18 - DNA, 21 bp, synthetic construct
  source 1..21: mol_type = other DNA; note = hsa-miR-192-F
tcggcaggctgacctatgaat

SEQ ID NO: 19 - DNA, 21 bp, synthetic construct
  source 1..21: mol_type = other DNA; note = hsa-miR-199-F
gccgagacagtagtctgcaca

SEQ ID NO: 20 - DNA, 21 bp, synthetic construct
  source 1..21: mol_type = other DNA; note = hsa-miR-21-F
tcggcaggtagcttatcagac

SEQ ID NO: 21 - DNA, 20 bp, synthetic construct
  source 1..20: mol_type = other DNA; note = hsa-miR-2115-F
catcagaattcatggaggct

SEQ ID NO: 22 - DNA, 21 bp, synthetic construct
  source 1..21: mol_type = other DNA; note = hsa-miR-221-F
gccgagagctacattgtctgc

SEQ ID NO: 23 - DNA, 21 bp, synthetic construct
  source 1..21: mol_type = other DNA; note = hsa-miR-223-F
tcggcaggtgtcagtttgtca

SEQ ID NO: 24 - DNA, 21 bp, synthetic construct
  source 1..21: mol_type = other DNA; note = hsa-miR-26-F
tcggcaggttcaagtaatcca

SEQ ID NO: 25 - DNA, 21 bp, synthetic construct
  source 1..21: mol_type = other DNA; note = hsa-miR-27-F
gccgagttcacagtggctaag

SEQ ID NO: 26 - DNA, 21 bp, synthetic construct
  source 1..21: mol_type = other DNA; note = hsa-miR-4499-F
gattgctctgcgtgcggaatc

SEQ ID NO: 27 - DNA, 21 bp, synthetic construct
  source 1..21: mol_type = other DNA; note = hsa-miR-801-F
gattgctctgcgtgcggaatc

SEQ ID NO: 28 - DNA, 21 bp, synthetic construct
  source 1..21: mol_type = other DNA; note = RNU6-1-F
aacaagcgcaaggatgacacg

SEQ ID NO: 29 - DNA, 18 bp, synthetic construct
  source 1..18: mol_type = other DNA; note = Universal Rp
cagtgcagggtccgaggt

SEQ ID NO: 30 - DNA, 49 bp, synthetic construct
  source 1..49: mol_type = other DNA; note = Universal RT primer
cagtgcagggtccgaggtcagagccacctgggcaattttttttttttvn

SEQ ID NO: 31 - DNA, 13 bp, synthetic construct
  source 1..13: mol_type = other DNA; note = Universal Taqman Probe
tgcccaggtggct